European Patent Application EP 4 653 456 A2, published November 26, 2025. Title: CHIMERIC ANTIGEN RECEPTORS TARGETING B-CELL MATURATION ANTIGEN. Applicant: THE UNITED STATES OF AMERICA, AS REPRESENTED BY THE SECRETARY, DEPARTMENT OF HEALTH AND HUMAN SERVICES. The sequence listing filed with the application follows.

SEQUENCE LISTING (12 sequences)

SEQ ID NO: 1 - DNA, 1512 bp, synthetic construct
  misc_feature 1..1512: note = Synthetic
  source 1..1512: mol_type = other DNA
atggccctgcctgtgacagctctgctgctgcccctggccctgctgctccatgccgccagacccgacatcgtgctgacccagagcccccccagcctggccatgtctctgggcaagagagccaccatcagctgccgggccagcgagagcgtgaccatcctgggcagccacctgatctactggtatcagcagaagcctggccagccccccaccctgctgatccagctggctagcaatgtgcagaccggcgtgcccgccagattcagcggcagcggcagcagaaccgacttcaccctgaccatcgaccccgtggaagaggacgacgtggccgtgtactactgcctgcagagccggaccatcccccggacctttggcggaggaacaaagctggaaatcaagggcagcaccagcggctccggcaagcctggctctggcgagggcagcacaaagggacagattcagctggtgcagagcggccctgagctgaagaaacccggcgagacagtgaagatcagctgcaaggcctccggctacaccttccggcactacagcatgaactgggtgaaacaggcccctggcaagggcctgaagtggatgggccggatcaacaccgagagcggcgtgcccatctacgccgacgacttcaagggcagattcgccttcagcgtggaaaccagcgccagcaccgcctacctggtgatcaacaacctgaaggacgaggataccgccagctacttctgcagcaacgactacctgtacagcctggacttctggggccagggcaccgccctgaccgtgtccagcttcgtgcctgtgttcctgcccgccaagcccaccaccacccctgcccctagacctcccaccccagccccaacaatcgccagccagcctctgtccctgcggcccgaagcctgtagacctgctgccggcggagccgtgcacaccagaggcctggatttcgcctgcgacatctacatctgggcccctctggccggcacctgtggcgtgctgctgctgagcctggtgatcaccctgtactgcaaccaccggaacagaagcaagcggagccggctgctgcacagcgactacatgaacatgaccccaagacggcctggccccacccggaagcactaccagccttacgcccctcccagagacttcgccgcctaccggtccagagtgaagttcagcagatccgccgacgcccctgcctaccagcagggacagaaccagctgtacaacgagctgaacctgggcagacgggaagagtacgacgtgctggacaagcggagaggccgggaccccgagatgggcggaaagcccagacggaagaacccccaggaaggcctgtataacgaactgcagaaagacaagatggccgaggcctacagcgagatcggcatgaagggcgagcggaggcgcggcaagggccacgatggcctgtaccagggcctgagcaccgccaccaaggacacctacgacgccctgcacatgcaggccctgccccccagatga

SEQ ID NO: 2 - DNA, 1512 bp, synthetic construct
  misc_feature 1..1512: note = Synthetic
  source 1..1512: mol_type = other DNA
atggccctgcctgtgacagctctgctcctccctctggccctgctgctccatgccgccagacccgacatcgtgctgacccagagcccccccagcctggccatgtctctgggcaagagagccaccatcagctgccgggccagcgagagcgtgaccatcctgggcagccacctgatccactggtatcagcagaagcccggccagccccccaccctgctgatccagctcgccagcaatgtgcagaccggcgtgcccgccagattcagcggcagcggcagcagaaccgacttcaccctgaccatcgaccccgtggaagaggacgacgtggccgtgtactactgcctgcagagccggaccatcccccggacctttggcggaggcaccaaactggaaatcaagggcagcaccagcggctccggcaagcctggctctggcgagggcagcacaaagggacagattcagctggtgcagagcggccctgagctgaagaaacccggcgagacagtgaagatcagctgcaaggcctccggctacaccttcaccgactacagcatcaactgggtgaaaagagcccctggcaagggcctgaagtggatgggctggatcaacaccgagacaagagagcccgcctacgcctacgacttccggggcagattcgccttcagcctggaaaccagcgccagcaccgcctacctgcagatcaacaacctgaagtacgaggacaccgccacctacttttgcgccctggactacagctacgccatggactactggggccagggcaccagcgtgaccgtgtccagcttcgtgcccgtgttcctgcccgccaaacctaccaccacccctgcccctagacctcccaccccagccccaacaatcgccagccagcctctgtctctgcggcccgaagcctgtagacctgctgccggcggagccgtgcacaccagaggcctggacttcgcctgcgacatctacatctgggcccctctggccggcacctgtggcgtgctgctgctgagcctggtgatcaccctgtactgcaaccaccggaacagaagcaagcggagccggctgctgcacagcgactacatgaacatgaccccaagacggcctggccccacccggaagcactaccagccttacgcccctcccagagacttcgccgcctaccggtccagagtgaagttcagcagatccgccgacgcccctgcctaccagcagggacagaaccagctgtacaacgagctgaacctgggcagacgggaagagtacgacgtgctggacaagcggagaggccgggaccccgagatgggcggaaagcccagacggaagaacccccaggaaggcctgtataacgaactgcagaaagacaagatggccgaggcctacagcgagatcggcatgaagggcgagcggaggcgcggcaagggccacgatggcctgtaccagggcctgagcaccgccaccaaggacacctacgacgccctgcacatgcaggccctgccccccagatga

SEQ ID NO: 3 - DNA, 1512 bp, synthetic construct
  misc_feature 1..1512: note = Synthetic
  source 1..1512: mol_type = other DNA
atggctctgcctgtgacagctctgctgctgcctctggccctgctgctgcatgccgccagacctgatatcgtgctgacccagagccctcccagcctggccatgtctctgggcaagagagccaccatcagctgcagagccagcgagagcgtgaccatcctgggcagccacctgatctactggtatcagcagaagcccggccagccccccacactgctgattcagctggcctccaatgtgcagaccggcgtgccagccagattttccggcagcggcagcagaaccgacttcaccctgaccatcgaccccgtggaagaggacgacgtggccgtgtactactgcctgcagagcagaaccatcccccggacctttggcggaggcaccaagctggaaatcaagggcagcaccagcggctccggcaagcctggatctggcgagggatctaccaagggacagatccagctggtgcagagcggccctgagctgaagaaacccggcgagacagtgaagatctcctgcaaggccagcggctacaccttcacccactacagcatgaactgggtcaagcaggcccctggcaagggcctgaagtggatgggccggatcaacaccgagacaggcgagcccctgtacgccgacgactttaagggcagattcgccttcagcctggaaaccagcgccagcaccgcctacctcgtgatcaacaacctgaagaacgaggacaccgccacctttttctgctccaacgactacctgtacagctgcgactactggggccagggcaccaccctgacagtgtctagcttcgtgcccgtgttcctgcccgccaagcctacaacaacccctgcccctagacctcccaccccagcccctacaattgcctctcagcctctgagcctgaggcccgaggcttgtagaccagctgctggcggagccgtgcacaccagaggactggatttcgcctgcgacatctacatctgggcccctctggccggcacctgtggcgtgctgctgctgagcctggtgatcaccctgtactgcaaccaccggaacagaagcaagcggagccggctgctgcacagcgactacatgaacatgaccccaagacggcctggccccacccggaagcactaccagccttacgcccctcccagagacttcgccgcctaccggtccagagtgaagttcagcagatccgccgacgcccctgcctaccagcagggacagaaccagctgtacaacgagctgaacctgggcagacgggaagagtacgacgtgctggacaagcggagaggccgggaccccgagatgggcggaaagcccagacggaagaacccccaggaaggcctgtataacgaactgcagaaagacaagatggccgaggcctacagcgagatcggcatgaagggcgagcggaggcgcggcaagggccacgatggcctgtaccagggcctgagcaccgccaccaaggacacctacgacgccctgcacatgcaggccctgccccccagatga

SEQ ID NO: 4 - protein, 503 aa, synthetic construct
  REGION 1..503: note = Synthetic
MALPVTALLLPLALLLHAARPDIVLTQSPPSLAMSLGKRATISCRASESVTILGSHLIYWYQQKPGQPPTLLIQLASNVQTGVPARFSGSGSRTDFTLTIDPVEEDDVAVYYCLQSRTIPRTFGGGTKLEIKGSTSGSGKPGSGEGSTKGQIQLVQSGPELKKPGETVKISCKASGYTFRHYSMNWVKQAPGKGLKWMGRINTESGVPIYADDFKGRFAFSVETSASTAYLVINNLKDEDTASYFCSNDYLYSLDFWGQGTALTVSSFVPVFLPAKPTTTPAPRPPTPAPTIASQPLSLRPEACRPAAGGAVHTRGLDFACDIYIWAPLAGTCGVLLLSLVITLYCNHRNRSKRSRLLHSDYMNMTPRRPGPTRKHYQPYAPPRDFAAYRSRVKFSRSADAPAYQQGQNQLYNELNLGRREEYDVLDKRRGRDPEMGGKPRRKNPQEGLYNELQKDKMAEAYSEIGMKGERRRGKGHDGLYQGLSTATKDTYDALHMQALPPR

SEQ ID NO: 5 - protein, 503 aa, synthetic construct
  REGION 1..503: note = Synthetic
MALPVTALLLPLALLLHAARPDIVLTQSPPSLAMSLGKRATISCRASESVTILGSHLIHWYQQKPGQPPTLLIQLASNVQTGVPARFSGSGSRTDFTLTIDPVEEDDVAVYYCLQSRTIPRTFGGGTKLEIKGSTSGSGKPGSGEGSTKGQIQLVQSGPELKKPGETVKISCKASGYTFTDYSINWVKRAPGKGLKWMGWINTETREPAYAYDFRGRFAFSLETSASTAYLQINNLKYEDTATYFCALDYSYAMDYWGQGTSVTVSSFVPVFLPAKPTTTPAPRPPTPAPTIASQPLSLRPEACRPAAGGAVHTRGLDFACDIYIWAPLAGTCGVLLLSLVITLYCNHRNRSKRSRLLHSDYMNMTPRRPGPTRKHYQPYAPPRDFAAYRSRVKFSRSADAPAYQQGQNQLYNELNLGRREEYDVLDKRRGRDPEMGGKPRRKNPQEGLYNELQKDKMAEAYSEIGMKGERRRGKGHDGLYQGLSTATKDTYDALHMQALPPR

SEQ ID NO: 6 - protein, 503 aa, synthetic construct
  REGION 1..503: note = Synthetic
MALPVTALLLPLALLLHAARPDIVLTQSPPSLAMSLGKRATISCRASESVTILGSHLIYWYQQKPGQPPTLLIQLASNVQTGVPARFSGSGSRTDFTLTIDPVEEDDVAVYYCLQSRTIPRTFGGGTKLEIKGSTSGSGKPGSGEGSTKGQIQLVQSGPELKKPGETVKISCKASGYTFTHYSMNWVKQAPGKGLKWMGRINTETGEPLYADDFKGRFAFSLETSASTAYLVINNLKNEDTATFFCSNDYLYSCDYWGQGTTLTVSSFVPVFLPAKPTTTPAPRPPTPAPTIASQPLSLRPEACRPAAGGAVHTRGLDFACDIYIWAPLAGTCGVLLLSLVITLYCNHRNRSKRSRLLHSDYMNMTPRRPGPTRKHYQPYAPPRDFAAYRSRVKFSRSADAPAYQQGQNQLYNELNLGRREEYDVLDKRRGRDPEMGGKPRRKNPQEGLYNELQKDKMAEAYSEIGMKGERRRGKGHDGLYQGLSTATKDTYDALHMQALPPR

SEQ ID NO: 7 - protein, 18 aa, synthetic construct
  REGION 1..18: note = Synthetic
GSTSGSGKPGSGEGSTKG

SEQ ID NO: 8 - protein, 507 aa, synthetic construct
  REGION 1..507: note = Synthetic
MLLLVTSLLLCELPHPAFLLIPDIVLTQSPPSLAMSLGKRATISCRASESVTILGSHLIHWYQQKPGQPPTLLIQLASNVQTGVPARFSGSGSRTDFTLTIDPVEEDDVAVYYCLQSRTIPRTFGGGTKLEIKGSTSGSGKPGSGEGSTKGQIQLVQSGPELKKPGETVKISCKASGYTFTDYSINWVKRAPGKGLKWMGWINTETREPAYAYDFRGRFAFSLETSASTAYLQINNLKYEDTATYFCALDYSYAMDYWGQGTSVTVSSAAAFVPVFLPAKPTTTPAPRPPTPAPTIASQPLSLRPEACRPAAGGAVHTRGLDFACDIYIWAPLAGTCGVLLLSLVITLYCNHRNRSKRSRLLHSDYMNMTPRRPGPTRKHYQPYAPPRDFAAYRSRVKFSRSADAPAYQQGQNQLYNELNLGRREEYDVLDKRRGRDPEMGGKPRRKNPQEGLYNELQKDKMAEAYSEIGMKGERRRGKGHDGLYQGLSTATKDTYDALHMQALPPR

SEQ ID NO: 9 - protein, 506 aa, synthetic construct
  REGION 1..506: note = Synthetic
MALPVTALLLPLALLLHAARPDIVLTQSPPSLAMSLGKRATISCRASESVTILGSHLIHWYQQKPGQPPTLLIQLASNVQTGVPARFSGSGSRTDFTLTIDPVEEDDVAVYYCLQSRTIPRTFGGGTKLEIKGSTSGSGKPGSGEGSTKGQIQLVQSGPELKKPGETVKISCKASGYTFTDYSINWVKRAPGKGLKWMGWINTETREPAYAYDFRGRFAFSLETSASTAYLQINNLKYEDTATYFCALDYSYAMDYWGQGTSVTVSSAAAFVPVFLPAKPTTTPAPRPPTPAPTIASQPLSLRPEACRPAAGGAVHTRGLDFACDIYIWAPLAGTCGVLLLSLVITLYCNHRNRSKRSRLLHSDYMNMTPRRPGPTRKHYQPYAPPRDFAAYRSRVKFSRSADAPAYQQGQNQLYNELNLGRREEYDVLDKRRGRDPEMGGKPRRKNPQEGLYNELQKDKMAEAYSEIGMKGERRRGKGHDGLYQGLSTATKDTYDALHMQALPPR

SEQ ID NO: 10 - protein, 512 aa, synthetic construct
  REGION 1..512: note = Synthetic
MALPVTALLLPLALLLHAARPDIVLTQSPPSLAMSLGKRATISCRASESVTILGSHLIHWYQQKPGQPPTLLIQLASNVQTGVPARFSGSGSRTDFTLTIDPVEEDDVAVYYCLQSRTIPRTFGGGTKLEIKGSTSGSGKPGSGEGSTKGQIQLVQSGPELKKPGETVKISCKASGYTFTDYSINWVKRAPGKGLKWMGWINTETREPAYAYDFRGRFAFSLETSASTAYLQINNLKYEDTATYFCALDYSYAMDYWGQGTSVTVSSAAAFVPVFLPAKPTTTPAPRPPTPAPTIASQPLSLRPEACRPAAGGAVHTRGLDFACDIYIWAPLAGTCGVLLLSLVITLYCNHRNRFSVVKRGRKKLLYIFKQPFMRPVQTTQEEDGCSCRFPEEEEGGCELRVKFSRSADAPAYQQGQNQLYNELNLGRREEYDVLDKRRGRDPEMGGKPRRKNPQEGLYNELQKDKMAEAYSEIGMKGERRRGKGHDGLYQGLSTATKDTYDALHMQALPPR

SEQ ID NO: 11 - protein, 502 aa, synthetic construct
  REGION 1..502: note = Synthetic
MALPVTALLLPLALLLHAARPDIVLTQSPPSLAMSLGKRATISCRASESVTILGSHLIHWYQQKPGQPPTLLIQLASNVQTGVPARFSGSGSRTDFTLTIDPVEEDDVAVYYCLQSRTIPRTFGGGTKLEIKGSTSGSGKPGSGEGSTKGQIQLVQSGPELKKPGETVKISCKASGYTFTDYSINWVKRAPGKGLKWMGWINTETREPAYAYDFRGRFAFSLETSASTAYLQINNLKYEDTATYFCALDYSYAMDYWGQGTSVTVSSAAAFVPVFLPAKPTTTPAPRPPTPAPTIASQPLSLRPEACRPAAGGAVHTRGLDFACDIYIWAPLAGTCGVLLLSLVITLYCNHRNRRDQRLPPDAHKPPGGGSFRTPIQEEQADAHSTLAKIRVKFSRSADAPAYQQGQNQLYNELNLGRREEYDVLDKRRGRDPEMGGKPRRKNPQEGLYNELQKDKMAEAYSEIGMKGERRRGKGHDGLYQGLSTATKDTYDALHMQALPPR

SEQ ID NO: 12 - protein, 549 aa, synthetic construct
  REGION 1..549: note = Synthetic
MALPVTALLLPLALLLHAARPDIVLTQSPPSLAMSLGKRATISCRASESVTILGSHLIHWYQQKPGQPPTLLIQLASNVQTGVPARFSGSGSRTDFTLTIDPVEEDDVAVYYCLQSRTIPRTFGGGTKLEIKGSTSGSGKPGSGEGSTKGQIQLVQSGPELKKPGETVKISCKASGYTFTDYSINWVKRAPGKGLKWMGWINTETREPAYAYDFRGRFAFSLETSASTAYLQINNLKYEDTATYFCALDYSYAMDYWGQGTSVTVSSAAAFVPVFLPAKPTTTPAPRPPTPAPTIASQPLSLRPEACRPAAGGAVHTRGLDFACDIYIWAPLAGTCGVLLLSLVITLYCNHRNRFSVVKRGRKKLLYIFKQPFMRPVQTTQEEDGCSCRFPEEEEGGCELRRDQRLPPDAHKPPGGGSFRTPIQEEQADAHSTLAKIRVKFSRSADAPAYQQGQNQLYNELNLGRREEYDVLDKRRGRDPEMGGKPRRKNPQEGLYNELQKDKMAEAYSEIGMKGERRRGKGHDGLYQGLSTATKDTYDALHMQALPPR